European Patent Application EP 4 183 859 A1, published May 24, 2023. Title: AMYLASE-CONTAINING DETERGENT COMPOSITION. Applicant: KAO CORPORATION. The sequence listing filed with the application follows.

SEQUENCE LISTING (48 sequences)

SEQ ID NO: 1 - DNA, 1458 bp, Bacillus flexus DE0178
  CDS (1)..(1455): Codon-optimized oligonucleotide
gcagctcaaaacggtacgatgatgcagtactttgaatggtatgtaccgaatgatggtcagcattggaatcgtctgcggaacgatgcagcctacttgaaatccatcggtgtgtcagctgtttggacacctcctgcttacaaaggcacaagccagaacgatgttggctatggagcatatgacctgtacgatttaggagaattcaaccagaaaggcactattcgcaccaaatatggaacgaaagctgaactgaaaagcgcggtaaacactctcaagtctaatgggattcaagtgtatggagatgtcgtcatgaatcataaaggcggtgccgattacacagagaatgtaacagctgtggaagtcaatccgagcaatcgcaatcaagaaacatccgatgagtatacgatccaagcatggacaggattcaacttccctgggcgaggcacaacccatagtccgtttaagtggcagtggtatcattttgatggaactgactgggatcagtctcggaatgcgagcagaatcttcaaatttcgtgggacaggaaaagcatgggattgggaagtatcatcggagaatgggaattacgactatcttatgtacgccgatttagactttgatcatcctgatgttggaaatgagatgaagaattggggcgtgtggtacgcgaatgaagttggcttggacggatttaggctggatgcggttaagcacataaagcatagctatctgggcgattgggtgaaccatgtcagaactaagacgggaaaagagatgtttacagttgctgaatattggcaaaacgacgtcaatgccattaataactatttagccaaagtgaactataatcactctgtctttgatgcgcctttgcattacaactttcactatgcaagccagtcaggaggtaactacgacatgcgtaacttattgaacggcacagtcgtggctgctcatccgacaaaagcagttacccttgtcgaaaatcatgacagtcaaccgggacaatctctggagtcagtcgttcaaccgtggtttaagccccttgcctatgcgtttatcctcacacgagcagaaggttatccaagtatcttttatggggatatgtatgggactaagggaaactcatcgtacgaaattccagcactcaaaaccaaaattgaaccgttactgaaagcacgcaaggattatgcctatggtacgcagcacaactatatggaccactgggatgttataggttggaccagagaaggtgactccacgaaagaaaaatctggccttgcgacgcttgtgacagacggggcaggcgggtctaaatggatgtatgtaggcaaacagaatgctggcgaagtttggtatgacatcacaggcaatagaacggataaaatcaccattaatacagatggctggggaaacttccaagtaaacggaggctcagtctccgtgtacgttcaacagtaa

SEQ ID NO: 2 - protein, 485 aa, Bacillus flexus DE0178
AAQNGTMMQYFEWYVPNDGQHWNRLRNDAAYLKSIGVSAVWTPPAYKGTSQNDVGYGAYDLYDLGEFNQKGTIRTKYGTKAELKSAVNTLKSNGIQVYGDVVMNHKGGADYTENVTAVEVNPSNRNQETSDEYTIQAWTGFNFPGRGTTHSPFKWQWYHFDGTDWDQSRNASRIFKFRGTGKAWDWEVSSENGNYDYLMYADLDFDHPDVGNEMKNWGVWYANEVGLDGFRLDAVKHIKHSYLGDWVNHVRTKTGKEMFTVAEYWQNDVNAINNYLAKVNYNHSVFDAPLHYNFHYASQSGGNYDMRNLLNGTVVAAHPTKAVTLVENHDSQPGQSLESVVQPWFKPLAYAFILTRAEGYPSIFYGDMYGTKGNSSYEIPALKTKIEPLLKARKDYAYGTQHNYMDHWDVIGWTREGDSTKEKSGLATLVTDGAGGSKWMYVGKQNAGEVWYDITGNRTDKITINTDGWGNFQVNGGSVSVYVQQ

SEQ ID NO: 3 - DNA, 1458 bp, Bacillus sp. RU2C
  CDS (1)..(1455): Codon-optimized oligonucleotide
gcagctcaaaacggtacgatgatgcagtactttgaatggtatgtaccgaatgatggtcagcattggaatcgtctgcggaacgatgcagcctacttgaaatccatcggtgtgtcagctgtttggacacctcctgcttacaaaggcacaagccagaacgatgttggctatggagcatatgacctgtacgatttaggagaattcaaccagaaaggcactattcgcaccaaatatggaacgaaagctgaactgaaaagcgcggtatcgactctcaagtctaatgggattcaagtgtatggagatgtcgtcatgaatcataaaggcggtgccgattacacagagaatgtaacagctgtggaagtcaatccgagcaatcgcaatcaagaaacatccgatgagtatacgatccaagcatggacaggattcaacttccctgggcgaggcacaacccatagtccgtttaagtggcagtggtatcattttgatggaactgactgggatcagtctcggaatgcgagcagaatcttcaaatttcgtgggacaggaaaagtttgggattgggaagtatcatcggagaatgggaattacgactatcttatgtacgccgatttagactttgatcatcctgatgttggaaatgagatgaagaattggggcgtgtggtacgcgaatgaagttggcttggacggatttaggctggatgcggttaagcacataaagcatagctatctgggcgattgggtgaaccatgtcagaactaagacgggaaaagagatgtttacagttgctgaatattggcaaaacgacgtcaatgccattaataactatttagccaaagtgaactataatcactctgtctttgatgcgcctttgcattacaactttcactatgcaagccagtcaggaggtaactacgacatgcgtaacttattgaacggcacagtcgtggctgctcatccgacaaaagcagttacccttgtcgaaaatcatgacagtcaaccgggacaatctctggagtcagtcgttcaaccgtggtttaagccccttgcctatgcgtttatcctcacacgagcagaaggttatccaagtatcttttatggggatatgtatgggactaagggaaactcatcgtacgaaattccagcactcaaaaccaaaattgaaccgttactgaaagcacgcaaggattatgcctatggtacgcagcacaactatatggaccactgggatgttataggttggaccagagaaggtgactccacgaaagaaaaatctggccttgcgacgcttgtgacagacggggcaggcgggtctaaatggatgtatgtaggcaaacagaatgctggcgaagtttggtatgacatcacaggcaatagaacggataaaatcaccattaatacagatggctggggaaacttccaagtaaacggaggctcagtctccgtgtacgttcaacagtaa

SEQ ID NO: 4 - protein, 485 aa, Bacillus sp. RU2C
AAQNGTMMQYFEWYVPNDGQHWNRLRNDAAYLKSIGVSAVWTPPAYKGTSQNDVGYGAYDLYDLGEFNQKGTIRTKYGTKAELKSAVSTLKSNGIQVYGDVVMNHKGGADYTENVTAVEVNPSNRNQETSDEYTIQAWTGFNFPGRGTTHSPFKWQWYHFDGTDWDQSRNASRIFKFRGTGKVWDWEVSSENGNYDYLMYADLDFDHPDVGNEMKNWGVWYANEVGLDGFRLDAVKHIKHSYLGDWVNHVRTKTGKEMFTVAEYWQNDVNAINNYLAKVNYNHSVFDAPLHYNFHYASQSGGNYDMRNLLNGTVVAAHPTKAVTLVENHDSQPGQSLESVVQPWFKPLAYAFILTRAEGYPSIFYGDMYGTKGNSSYEIPALKTKIEPLLKARKDYAYGTQHNYMDHWDVIGWTREGDSTKEKSGLATLVTDGAGGSKWMYVGKQNAGEVWYDITGNRTDKITINTDGWGNFQVNGGSVSVYVQQ

SEQ ID NO: 5 - DNA, 1458 bp, Bacillus sp. CGMCC 1.16541
  CDS (1)..(1455): Codon-optimized oligonucleotide
gcaaaacaaaatgggacgatgatgcagtattttgaatggtatttaccaaacgatggtcaacactggaacagacttagaacagacgctacgtatttaaaaagcattggagtttctgcggtttggacacctccggcttataagggcactagtcaaaacgatgttgggtatggagcgtatgatctttacgacctgggagaatttaatcaaaaagggacggtacgaacaaaatatggaacaaaagcagaattaaagagcgcggtatctactcttaaagctaatggtatccaggtttatggagatgtcgttatgaatcacaaggggggcgcagattataccgagaatgtaacagctgtagaagttaatccaagtaaccgcaaccaagaaacaagcggcgattatatgattcaagcgtggacaggatttaattttccaggccgagggaatacgcattcgtcatttaaatggaaatggtatcattttgatggaacggattgggatcaatcaagaaatgcaagtagaattttcaaatttcgaggtacagggaaggcgtgggattgggaagtatcaacggaaaacggcaattatgactatttaatgtacgctgatgtggattttgaacatccggacgtggcaaacgaaatgaagaattggggcgtgtggtatgcaaatgaagttggattagacggattccggttagatgctgttaagcacataaaacacaattatcttggagattgggtgaaccatgttagaacgagaacaggtaaagaaatgtttacagttgcagaatattggcaaaatgatgtaaacgctattaataactatctggcaaaggtcaattataaccatagtgttttcgacgctcctttacattataattttcattacgcttcacaatcaggtggcaattacgatatgcgaaacttattaaatggaacggtggtggcgacgcatcctacgaaagcagtcacgctcgtagaaaatcatgactcacaaccaggacaatcgcttgaatcagtcgtccaatcgtggtttaaacctcttgcttacgcttttattttaacccgtgcacaaggctatccgtcagttttttatggagatatgtatggaacaaatggtaattcatcttatgagatccctgcccttaaaacaaaactcgaacctttattgaaagctcgtaaagactatgcatacggtacgcagcacaattatatggaccactgggatgttattggttggacacgcgagggggacgggacaaaagcaaaatcggggcttgcgactttaataacggatggaccaggaggcagcaaatggatgtatgtcggaaaacaaaacgcaggcgaagtctggggagatttaacaggaaatagaggggataaagtgaccattaacgcggatggctggggacagttttatgtaaatggaggatccgtcagtgtgtatgtacaacaataa

SEQ ID NO: 6 - protein, 485 aa, Bacillus sp. CGMCC 1.16541
AKQNGTMMQYFEWYLPNDGQHWNRLRTDATYLKSIGVSAVWTPPAYKGTSQNDVGYGAYDLYDLGEFNQKGTVRTKYGTKAELKSAVSTLKANGIQVYGDVVMNHKGGADYTENVTAVEVNPSNRNQETSGDYMIQAWTGFNFPGRGNTHSSFKWKWYHFDGTDWDQSRNASRIFKFRGTGKAWDWEVSTENGNYDYLMYADVDFEHPDVANEMKNWGVWYANEVGLDGFRLDAVKHIKHNYLGDWVNHVRTRTGKEMFTVAEYWQNDVNAINNYLAKVNYNHSVFDAPLHYNFHYASQSGGNYDMRNLLNGTVVATHPTKAVTLVENHDSQPGQSLESVVQSWFKPLAYAFILTRAQGYPSVFYGDMYGTNGNSSYEIPALKTKLEPLLKARKDYAYGTQHNYMDHWDVIGWTREGDGTKAKSGLATLITDGPGGSKWMYVGKQNAGEVWGDLTGNRGDKVTINADGWGQFYVNGGSVSVYVQQ

SEQ ID NO: 7 - DNA, 1458 bp, Bacillus sp. YR288
  CDS (1)..(1455): Codon-optimized oligonucleotide
gcagctcaaaacggtacgatgatgcagtactttgaatggtatgtaccgaatgatggtcagcattggaatcgtctgcggaacgatgcagcctacttgaaatccatcggtgtgtcagctatctggacacctcctgcttacaaaggcacaagccagaacgatgttggctatggagcatatgacctgtacgatttaggagaattcaaccagaaaggcactattcgcaccaaatatggaacgaaagctgaactgaaaagcgcggtatcgactctcaagtctaatgggattcaagtgtatggagatgtcgtcatgaatcataaaggcggtgccgattacacagagaatgtaacagctgtggaagtcaatccgagcaatcgcaatcaagaaacatccgatgagtatacgatccaagcatggacaggattcaacttccctgggcgaggcacaacccatagtccgtttaagtggcagtggtatcattttgatggaactgactgggatcagtctcggaatgcgagcagaatcttcaaatttcgtgggacaggaaaagcatgggattgggaagtatcatcggagaatgggaattacgactatcttatgtacgccgatttagactttgatcatcctgatgttagaaatgagatgaagaattggggcgtgtggtacgcgaatgaagttggcttggacggatttaggctggatgcggttaagcacataaagcatagctatctgggcgattgggtgaaccatgtcagaactaagacgggaaaagagatgtttacagttgctgaatattggcaaaacgacgtcaatgccattaataactatttagccaaagtgaactataatcactctgtctttgatgcgcctttgcattacaactttcactatgcaagccagtcaggaggtaactacgacatgcgtaacttattgaacggcacagtcgtggctgctcatccgacaaaagcagttacccttgtcgaaaatcatgacagtcaaccgggacaatctctggagtcagtcgttcaaccgtggtttaagccccttgcctatgcgtttatcctcacacgagcagaaggttatccaagtatcttttatggggatatgtatgggactaagggaaactcatcgtacgaaattccagcactcaaaaccaaaattgaaccgttactgaaagcacgcaaggattatgcctatggtacgcagcacaactatatggaccactgggatgttataggttggaccagagaaggtgactccacgaaagaaaaatctggccttgcgacgcttgtgacagacggggcaggcgggtctaaatggatgtatgtaggcaaacagaatgctggcgaagtttggtatgacatcacaggcaatagaacggataaaatcaccattaatacagatggctggggaaacttccaagtaaacggaggctcagtctccgtgtacgttcaacagtaa

SEQ ID NO: 8 - protein, 485 aa, Bacillus sp. YR288
AAQNGTMMQYFEWYVPNDGQHWNRLRNDAAYLKSIGVSAIWTPPAYKGTSQNDVGYGAYDLYDLGEFNQKGTIRTKYGTKAELKSAVSTLKSNGIQVYGDVVMNHKGGADYTENVTAVEVNPSNRNQETSDEYTIQAWTGFNFPGRGTTHSPFKWQWYHFDGTDWDQSRNASRIFKFRGTGKAWDWEVSSENGNYDYLMYADLDFDHPDVRNEMKNWGVWYANEVGLDGFRLDAVKHIKHSYLGDWVNHVRTKTGKEMFTVAEYWQNDVNAINNYLAKVNYNHSVFDAPLHYNFHYASQSGGNYDMRNLLNGTVVAAHPTKAVTLVENHDSQPGQSLESVVQPWFKPLAYAFILTRAEGYPSIFYGDMYGTKGNSSYEIPALKTKIEPLLKARKDYAYGTQHNYMDHWDVIGWTREGDSTKEKSGLATLVTDGAGGSKWMYVGKQNAGEVWYDITGNRTDKITINTDGWGNFQVNGGSVSVYVQQ

SEQ ID NO: 9 - DNA, 1458 bp, Bacillus sp. KSM-1378
  CDS (1)..(1455): Codon-optimized oligonucleotide
catcataatggcacaaacggaacaatgatgcagtattttgaatggcatttaccgaatgatggcaaccattggaatagactgcgcgatgatgcagcgaatcttaaaagcaaaggcattacagctgtttggatcccgccggcctggaaaggaacatctcaaaacgatgtgggctatggagcttacgatctgtacgatctgggcgaatttaatcagaaaggaacagtcagaacaaaatatggcacacgctctcaattacagggagccgtgacatcactgaaaaataacggcattcaagtctatggagatgttgtgatgaatcataaaggcggagcagatggcacagaaatggttaatgcggttgaagtgaacagaagcaatcgcaaccaggaaatttctggagaatatacaatcgaagcatggacaaaatttgattttccgggcagaggaaatacacattcaaactttaaatggcgctggtatcattttgatggcacagattgggatcaaagcagacaactgcagaacaaaatctacaaatttcgcggcacaggaaaagcttgggattgggaagtggatatcgaaaacggaaactacgattacctgatgtacgccgatattgatatggatcatccggaagtcatcaatgaactgagaaactggggcgtttggtacacaaacacacttaacctggatggatttcgcattgatgcggtcaaacatatcaaatactcatacacaagagattggctgacacatgttcgcaatacaacaggcaaaccgatgtttgcagtggcggaattttggaaaaacgatcttgctgccatcgaaaactacctgaacaaaacatcatggaatcatagcgtctttgatgttccgcttcattacaacctgtacaacgcttctaactcaggcggatattttgatatgagaaacatccttaacggctctgtcgttcagaaacatccgatccatgcagtgacatttgtcgataatcatgattcacaaccgggagaagcgctggaatcttttgtgcagtcatggtttaaaccgcttgcttatgccctgattcttacacgcgaacaaggctatccgagcgtgttttatggcgattattatggaattccgacacatggagtcccgagcatgaaatctaaaatcgatccgttactgcaagcaagacagacatatgcgtatggaacacagcatgattactttgatcatcatgatatcatcggctggacacgcgaaggagattcaagccatccgaattcaggccttgcaacaatcatgagcgatggaccgggcggaaacaaatggatgtatgttggcaaacataaagcgggacaagtgtggagagatattacaggcaatcgcagcggaacagtcacaatcaacgctgatggctggggaaattttacagttaacggcggagccgtctctgtttgggtgaaacagtaa

SEQ ID NO: 10 - protein, 485 aa, Bacillus sp. KSM-1378
HHNGTNGTMMQYFEWHLPNDGNHWNRLRDDAANLKSKGITAVWIPPAWKGTSQNDVGYGAYDLYDLGEFNQKGTVRTKYGTRSQLQGAVTSLKNNGIQVYGDVVMNHKGGADGTEMVNAVEVNRSNRNQEISGEYTIEAWTKFDFPGRGNTHSNFKWRWYHFDGTDWDQSRQLQNKIYKFRGTGKAWDWEVDIENGNYDYLMYADIDMDHPEVINELRNWGVWYTNTLNLDGFRIDAVKHIKYSYTRDWLTHVRNTTGKPMFAVAEFWKNDLAAIENYLNKTSWNHSVFDVPLHYNLYNASNSGGYFDMRNILNGSVVQKHPIHAVTFVDNHDSQPGEALESFVQSWFKPLAYALILTREQGYPSVFYGDYYGIPTHGVPSMKSKIDPLLQARQTYAYGTQHDYFDHHDIIGWTREGDSSHPNSGLATIMSDGPGGNKWMYVGKHKAGQVWRDITGNRSGTVTINADGWGNFTVNGGAVSVWVKQ

SEQ ID NO: 11 - DNA, 1458 bp, Bacillus sp. DSM12649
  CDS (1)..(1455): Codon-optimized oligonucleotide
catcataatggaacaaacggcacaatgatgcaatactttgaatggtatttaccgaacgatggaaaccattggaatagattacgcagcgatgcgtctaacctgaaagataaaggaatttcagctgtttggatcccgccggcatggaaaggagctagccaaaatgatgtgggctatggagcgtacgatctttacgatctgggagaatttaaccagaaaggcacaattcgcacaaaatatggcacaagaaatcaacttcaggcagcggtgaacgctttaaaatcaaatggaatccaagtctatggcgatgttgtgatgaatcataaaggcggagctgatgccacagaaatggtccgcgccgttgaagtgaacccgaataacagaaatcaggaagttagcggagaatacacaatcgaagcatggacaaaatttgattttccgggccgcggaaacacacattctaactttaaatggagatggtaccattttgatggcgttgattgggatcagtcaagaaaactgaacaaccgcatctacaaatttagaggcgatggaaaaggctgggattgggaagtggatacagaaaacggaaactacgattacctgatgtatgccgatatcgatatggatcatccggaagtcgttaacgaacttcgcaattggggcgtgtggtatacaaatacactgggacttgatggctttagaattgatgcggtcaaacatatcaaatatagctttacacgcgattggattaaccatgttagatctgcgacaggaaaaaatatgtttgcagtggcggaattttggaaaaatgatctgggcgctatcgaaaactaccttaacaaaacaaactggaaccattctgtctttgatgttccgctgcattacaacctttacaacgcgtcaaaaagcggcggaaactatgatatgcgccaaatttttaatggaacagtggtccagagacatccgatgcatgccgtgacatttgtcgataatcatgattctcaaccggaagaagcactggaatcatttgttgaagaatggtttaaaccgctggcttatgccttaacactgacacgcgaacagggatatccgagcgtgttttatggagattattatggcatcccgacacatggcgtcccggctatgaaatctaaaattgatccgatccttgaagctcgccaaaaatatgcctatggcagacagaacgattacctggatcatcataacatcatcggatggacaagagaaggcaacacagcacatccgaattcaggacttgcgacaattatgagcgatggcgctggcggaaacaaatggatgtttgtcggacgcaataaagcaggccaagtttggacagatattacaggaaacagagccggaacagtcacaatcaatgcagatggatggggcaactttagcgttaatggcggctcagtttcaatctgggtgaataaataa

SEQ ID NO: 12 - protein, 485 aa, Bacillus sp. DSM12649
HHNGTNGTMMQYFEWYLPNDGNHWNRLRSDASNLKDKGISAVWIPPAWKGASQNDVGYGAYDLYDLGEFNQKGTIRTKYGTRNQLQAAVNALKSNGIQVYGDVVMNHKGGADATEMVRAVEVNPNNRNQEVSGEYTIEAWTKFDFPGRGNTHSNFKWRWYHFDGVDWDQSRKLNNRIYKFRGDGKGWDWEVDTENGNYDYLMYADIDMDHPEVVNELRNWGVWYTNTLGLDGFRIDAVKHIKYSFTRDWINHVRSATGKNMFAVAEFWKNDLGAIENYLNKTNWNHSVFDVPLHYNLYNASKSGGNYDMRQIFNGTVVQRHPMHAVTFVDNHDSQPEEALESFVEEWFKPLAYALTLTREQGYPSVFYGDYYGIPTHGVPAMKSKIDPILEARQKYAYGRQNDYLDHHNIIGWTREGNTAHPNSGLATIMSDGAGGNKWMFVGRNKAGQVWTDITGNRAGTVTINADGWGNFSVNGGSVSIWVNK

SEQ ID NO: 13 - DNA, 1458 bp, Bacillus sp. SP722
  CDS (1)..(1455): Codon-optimized oligonucleotide
catcataatggcacaaacggaacaatgatgcaatattttgaatggcatctgccgaatgatggcaaccattggaatagactgcgcgatgatgcttctaaccttagaaatcgcggcattacagctatttggatcccgccggcctggaaaggaacatcacagaatgatgtcggctatggagcctatgatctgtatgatcttggcgaatttaaccaaaaaggaacagttcgcacaaaatatggaacaagatcacagttagaaagcgctatccatgccctgaaaaataacggcgttcaagtgtatggagatgttgtgatgaatcataaaggcggagcagatgcgacagaaaacgtgcttgctgtcgaagttaatccgaataaccgcaaccaggaaatttcaggcgattatacaatcgaagcctggacaaaatttgattttccgggccgcggaaacacatactcagattttaaatggagatggtaccattttgatggagtcgattgggatcaaagcagacaatttcagaaccgcatctacaaatttagaggcgatggaaaagcttgggattgggaagttgatagcgaaaatggcaactatgattatctgatgtatgccgatgtggatatggatcatccggaagtcgttaatgaacttagacgctggggcgaatggtacacaaacacactgaacctggatggatttagaatcgatgcggttaaacatatcaaatacagctttacacgcgattggttaacacatgttagaaatgcaacaggcaaagaaatgtttgctgtggccgaattttggaaaaacgatttaggagcgctggaaaactacctgaacaaaacaaactggaaccattctgtgtttgatgtcccgcttcattacaacctgtacaacgcatcaaacagcggcggaaattatgatatggcgaaactgcttaacggcacagtggtccaaaaacatccgatgcatgcagttacatttgtggataatcatgattctcaaccgggagaaagccttgaatcttttgtgcaggaatggtttaaaccgttagcatatgcgcttattttaacacgcgaacagggctatccgagcgtgttttatggcgattattatggaatcccgacacattctgtcccggcaatgaaagcgaaaattgatccgatccttgaagcacgccaaaattttgcgtatggaacacagcatgattactttgatcatcataacatcatcggctggacaagagaaggaaatacaacacatccgaactctggcttagcaacaattatgtcagatggaccgggcggagaaaaatggatgtatgtgggccaaaataaagcgggacaggtctggcatgatattacaggcaataaaccgggaacagtcacaatcaacgctgatggatgggccaattttagcgttaacggcggatctgtctcaatctgggttaaaagataa

SEQ ID NO: 14 - protein, 485 aa, Bacillus sp. SP722
HHNGTNGTMMQYFEWHLPNDGNHWNRLRDDASNLRNRGITAIWIPPAWKGTSQNDVGYGAYDLYDLGEFNQKGTVRTKYGTRSQLESAIHALKNNGVQVYGDVVMNHKGGADATENVLAVEVNPNNRNQEISGDYTIEAWTKFDFPGRGNTYSDFKWRWYHFDGVDWDQSRQFQNRIYKFRGDGKAWDWEVDSENGNYDYLMYADVDMDHPEVVNELRRWGEWYTNTLNLDGFRIDAVKHIKYSFTRDWLTHVRNATGKEMFAVAEFWKNDLGALENYLNKTNWNHSVFDVPLHYNLYNASNSGGNYDMAKLLNGTVVQKHPMHAVTFVDNHDSQPGESLESFVQEWFKPLAYALILTREQGYPSVFYGDYYGIPTHSVPAMKAKIDPILEARQNFAYGTQHDYFDHHNIIGWTREGNTTHPNSGLATIMSDGPGGEKWMYVGQNKAGQVWHDITGNKPGTVTINADGWANFSVNGGSVSIWVKR

SEQ ID NO: 15 - DNA, 1458 bp, Cytophaga sp.
  CDS (1)..(1455): Codon-optimized oligonucleotide
gccgccactaatgggacgatgatgcagtactttgaatggtacgttccgaatgatggccaacagtggaacaggctgagaacagacgcaccgtacttatcaagcgttggcattacggctgtctggacgccaccggcgtataagggtacttcacaagcggatgttggatacggaccatatgacttgtacgatttaggggagtttaaccagaaagggacagtacgcaccaaatatggaacaaaaggcgaactgaaaagcgccgtcaatacgctgcattccaatggaattcaggtctatggcgatgtggttatgaaccataaagcaggagcggactatactgagaatgttactgcagtggaagtgaatccatccaatcgaaaccaggaaacttcaggagaatacaacatacaggcgtggaccggctttaacttcccaggccgtggaacgacatatagcaactttaaatggcaatggtttcactttgatggtacagattgggatcaaagccgatcactctccaggatcttcaagtttcgcggtacaggcaaagcttgggattgggaggtgtcgtctgaaaacggcaattacgattaccttatgtatgcagatatcgactatgaccatcctgacgtcgttaatgagatgaagaaatggggagtatggtacgctaatgaagtaggtttagatgggtatcggttggatgccgtcaaacacatcaaattcagctttctcaaagattgggtcgataacgcgagagcagcaaccgggaaggagatgtttacagtgggtgaatattggcaaaatgacttaggagctcttaacaactatttggcgaaagtcaactataatcagtctctgtttgatgctccgcttcattacaacttctatgcggctagtacaggaggtgggtattatgacatgcgcaacattctgaataatacgctggttgcgtctaatcccacaaaagctgttaccctggtagaaaatcatgacacacaaccgggccagtctttggaatccacagtgcaaccgtggttcaaacctctcgcatatgcttttatcttaacacgctctggcggatatccctcagtgttctacggggatatgtatggcacaaagggaacgacgacacgggaaattcctgcactgaaatcgaagattgaacctcttcttaaggcacggaaagactatgcctatggcactcaacgtgattatattgacaaccctgacgtcattggctggacaagagagggagattcgaccaaagcgaaaagcggattagcaacggtaatcactgatggcccgggtggatctaagcgtatgtatgtcggtacgtcaaatgccggggaaatctggtacgatcttaccggcaatagaaccgataaaattacgataggcagtgatggttatgccacatttccggttaatggaggctcagtgagtgtatgggtgcaacagtaa

SEQ ID NO: 16 - protein, 485 aa, Cytophaga sp.
AATNGTMMQYFEWYVPNDGQQWNRLRTDAPYLSSVGITAVWTPPAYKGTSQADVGYGPYDLYDLGEFNQKGTVRTKYGTKGELKSAVNTLHSNGIQVYGDVVMNHKAGADYTENVTAVEVNPSNRNQETSGEYNIQAWTGFNFPGRGTTYSNFKWQWFHFDGTDWDQSRSLSRIFKFRGTGKAWDWEVSSENGNYDYLMYADIDYDHPDVVNEMKKWGVWYANEVGLDGYRLDAVKHIKFSFLKDWVDNARAATGKEMFTVGEYWQNDLGALNNYLAKVNYNQSLFDAPLHYNFYAASTGGGYYDMRNILNNTLVASNPTKAVTLVENHDTQPGQSLESTVQPWFKPLAYAFILTRSGGYPSVFYGDMYGTKGTTTREIPALKSKIEPLLKARKDYAYGTQRDYIDNPDVIGWTREGDSTKAKSGLATVITDGPGGSKRMYVGTSNAGEIWYDLTGNRTDKITIGSDGYATFPVNGGSVSVWVQQ

SEQ ID NO: 17 - DNA, 29 bp, Artificial Sequence
  Synthetic oligonucleotide
taatctattaaactagttatagggttatc

SEQ ID NO: 18 - DNA, 18 bp, Artificial Sequence
  Synthetic oligonucleotide
tgctgcaagagctgccgg

SEQ ID NO: 19 - DNA, 33 bp, Artificial Sequence
  Synthetic oligonucleotide
gcagctcttgcagcagcagctcaaaacggtacg

SEQ ID NO: 20 - DNA, 33 bp, Artificial Sequence
  Synthetic oligonucleotide
agtttaatagattactgttgaacgtacacggag

SEQ ID NO: 21 - DNA, 33 bp, Artificial Sequence; identical to SEQ ID NO: 19
  Synthetic oligonucleotide

SEQ ID NO: 22 - DNA, 33 bp, Artificial Sequence; identical to SEQ ID NO: 20
  Synthetic oligonucleotide

SEQ ID NO: 23 - DNA, 39 bp, Artificial Sequence
  Synthetic oligonucleotide
gcagctcttgcagcagcaaaacaaaatgggacgatgatg

SEQ ID NO: 24 - DNA, 37 bp, Artificial Sequence
  Synthetic oligonucleotide
agtttaatagattattgttgtacatacacactgacgg

SEQ ID NO: 25 - DNA, 33 bp, Artificial Sequence; identical to SEQ ID NO: 19
  Synthetic oligonucleotide

SEQ ID NO: 26 - DNA, 33 bp, Artificial Sequence; identical to SEQ ID NO: 20
  Synthetic oligonucleotide

SEQ ID NO: 27 - DNA, 35 bp, Artificial Sequence
  Synthetic oligonucleotide
gcagctcttgcagcacatcataatggcacaaacgg

SEQ ID NO: 28 - DNA, 35 bp, Artificial Sequence
  Synthetic oligonucleotide
agtttaatagattactgtttcacccaaacagagac

SEQ ID NO: 29 - DNA, 38 bp, Artificial Sequence
  Synthetic oligonucleotide
gcagctcttgcagcacatcataatggaacaaacggcac

SEQ ID NO: 30 - DNA, 41 bp, Artificial Sequence
  Synthetic oligonucleotide
tagtttaatagattatttattcacccagattgaaactgagc

SEQ ID NO: 31 - DNA, 38 bp, Artificial Sequence
  Synthetic oligonucleotide
gcagctcttgcagcacatcataatggcacaaacggaac

SEQ ID NO: 32 - DNA, 41 bp, Artificial Sequence
  Synthetic oligonucleotide
tagtttaatagattatcttttaacccagattgagacagatc

SEQ ID NO: 33 - DNA, 32 bp, Artificial Sequence
  Synthetic oligonucleotide
gcagctcttgcagcagccgccactaatgggac

SEQ ID NO: 34 - DNA, 34 bp, Artificial Sequence
  Synthetic oligonucleotide
agtttaatagattactgttgcacccatacactca

SEQ ID NO: 35 - protein, 483 aa, Bacillus amyloliquefaciens
VNGTLMQYFEWYTPNDGQHWKRLQNDAEHLSDIGITAVWIPPAYKGLSQSDNGYGPYDLYDLGEFQQKGTVRTKYGTKSELQDAIGSLHSRNVQVYGDVVLNHKAGADATEDVTAVEVNPANRNQETSEEYQIKAWTDFRFPGRGNTYSDFKWHWYHFDGADWDESRKISRIFKFRGEGKAWDWEVSSENGNYDYLMYADVDYDHPDVVAETKKWGIWYANELSLDGFRIDAAKHIKFSFLRDWVQAVRQATGKEMFTVAEYWQNNAGKLENYLNKTSFNQSVFDVPLHFNLQAASSQGGGYDMRRLLDGTVVSRHPEKAVTFVENHDTQPGQSLESTVQTWFKPLAYAFILTRESGYPQVFYGDMYGTKGTSPKEIPSLKDNIEPILKARKEYAYGPQHDYIDHPDVIGWTREGDSSAAKSGLAALITDGPGGSKRMYAGLKNAGETWYDITGNRSDTVKIGSDGWGEFHVNDGSVSIYVQK

SEQ ID NO: 36 - protein, 483 aa, Bacillus licheniformis
ANLNGTLMQYFEWYMPNDGQHWKRLQNDSAYLAEHGITAVWIPPAYKGTSQADVGYGAYDLYDLGEFHQKGTVRTKYGTKGELQSAIKSLHSRDINVYGDVVINHKGGADATEDVTAVEVDPADRNRVISGEHRIKAWTHFHFPGRGSTYSDFKWHWYHFDGTDWDESRKLNRIYKFQGKAWDWEVSNENGNYDYLMYADIDYDHPDVAAEIKRWGTWYANELQLDGFRLDAVKHIKFSFLRDWVNHVREKTGKEMFTVAEYWQNDLGALENYLNKTNFNHSVFDVPLHYQFHAASTQGGGYDMRKLLNSTVVSKHPLKAVTFVDNHDTQPGQSLESTVQTWFKPLAYAFILTRESGYPQVFYGDMYGTKGDSQREIPALKHKIEPILKARKQYAYGAQHDYFDHHDIVGWTREGDSSVANSGLAALITDGPGGAKRMYVGRQNAGETWHDITGNRSEPVVINSEGWGEFHVNGGSVSIYVQR

SEQ ID NO: 37 - protein, 485 aa, Artificial Sequence
  Designed peptide
HHDGTNGTIMQYFEWNVPNDGQHWNRLHNNAQNLKNAGITAIWIPPAWKGTSQNDVGYGAYDLYDLGEFNQKGTVRTKYGTKAELERAIRSLKANGIQVYGDVVMNHKGGADFTERVQAVEVNPQNRNQEVSGTYQIEAWTGFNFPGRGNQHSSFKWRWYHFDGTDWDQSRQLANRIYKFRGDGKAWDWEVDTENGNYDYLMYADVDMDHPEVINELNRWGVWYANTLNLDGFRLDAVKHIKFSFMRDWLGHVRGQTGKNLFAVAEYWKNDLGALENYLSKTNWTMSAFDVPLHYNLYQASNSSGNYDMRNLLNGTLVQRHPSHAVTFVDNHDTQPGEALESFVQGWFKPLAYATILTREQGYPQVFYGDYYGIPSDGVPSYRQQIDPLLKARQQYAYGTQHDYLDNQDVIGWTREGDSAHAGSGLATVMSDGPGGSKTMYVGTAHAGQVFKDITGNRTDTVTINSAGNGTFPCNGGSVSIWVKQ

SEQ ID NO: 38 - protein, 485 aa, Bacillus sp.
HHNGTNGTMMQYFEWYLPNDGNHWNRLNSDASNLKSKGITAVWIPPAWKGASQNDVGYGAYDLYDLGEFNQKGTVRTKYGTRSQLQAAVTSLKNNGIQVYGDVVMNHKGGADATEMVRAVEVNPNNRNQEVTGEYTIEAWTRFDFPGRGNTHSSFKWRWYHFDGVDWDQSRRLNNRIYKFRGHGKAWDWEVDTENGNYDYLMYADIDMDHPEVVNELRNWGVWYTNTLGLDGFRIDAVKHIKYSFTRDWINHVRSATGKNMFAVAEFWKNDLGAIENYLQKTNWNHSVFDVPLHYNLYNASKSGGNYDMRNIFNGTVVQRHPSHAVTFVDNHDSQPEEALESFVEEWFKPLAYALTLTREQGYPSVFYGDYYGIPTHGVPAMRSKIDPILEARQKYAYGKQNDYLDHHNIIGWTREGNTAHPNSGLATIMSDGAGGSKWMFVGRNKAGQVWSDITGNRTGTVTINADGWGNFSVNGGSVSIWVNK

SEQ ID NO: 39 - protein, 484 aa, Bacillus sp.
NTAPINETMMQYFEWDLPNDGTLWTKVKNEAANLSSLGITALWLPPAYKGTSQSDVGYGVYDLYDLGEFNQKGTIRTKYGTKTQYIQAIQAAKAAGMQVYADVVFNHKAGADGTEFVDAVEVDPSNRNQETSGTYQIQAWTKFDFPGRGNTYSSFKWRWYHFDGTDWDESRKLNRIYKFRSTGKAWDWEVDTENGNYDYLMFADLDMDHPEVVTELKNWGTWYVNTTNIDGFRLDAVKHIKYTFFPDWLTYVRNQTGKNLFAVGEFWSYDVNKLHNYITKTNGSMSLFDAPLHNNFYTASKSSGYFDMRYLLNNTLMKDQPSLAVTLVDNHDTQPGQSLQSWVEPWFKPLAYAFILTRQEGYPCVFYGDYYGIPKYNIPGLKSKIDPLLIARRDYAYGTQRDYIDHQDIIGWTREGIDTKPNSGLAALITDGPGGSKWMYVGKKHAGKVFYDLTGNRSDTVTINADGWGEFKVNGGSVSIWVAK

SEQ ID NO: 40 - protein, 483 aa, Bacillus licheniformis [sequence omitted]

SEQ ID NO: 41 - protein, 485 aa, Bacillus sp.
HHDGTNGTIMQYFEWNVPNDGQHWNRLHNNAQNLKNAGITAIWIPPAWKGTSQNDVGYGAYDLYDLGEFNQKGTVRTKYGTKAELERAIRSLKANGIQVYGDVVMNHKGGADFTERVQAVEVNPQNRNQEVSGTYQIEAWTGFNFPGRGNQHSSFKWRWYHFDGTDWDQSRQLANRIYKFRGDGKAWDWEVDTENGNYDYLMYADVDMDHPEVINELNRWGVWYANTLNLDGFRLDAVKHIKFSFMRDWLGHVRGQTGKNLFAVAEYWKNDLGALENYLSKTNWTMSAFDVPLHYNLYQASNSSGNYDMRNLLNGTLVQRHPSHAVTFVDNHDTQPGEALESFVQGWFKPLAYATILTREQGYPQVFYGDYYGIPSDGVPSYRQQIDPLLKARQQYAYGRQHDYFDHWDVIGWTREGNASHPNSGLATIMSDGPGGSKWMYVGRQKAGEVWHDMTGNRSGTVTINQDGWGHFFVNGGSVSVWVKR

SEQ ID NO: 42 - protein, 269 aa, Bacillus clausii
AQSVPWGISRVQAPAAHNRGLTGSGVKVAVLDTGISTHPDLNIRGGASFVPGEPSTQDGNGHGTHVAGTIAALNNSIGVLGVAPSAELYAVKVLGASGSGSVSSIAQGLEWAGNNGMHVANLSLGSPSPSATLEQAVNSATSRGVLVVAASGNSGAGSISYPARYANAMAVGATDQNNNRASFSQYGAGLDIVAPGVNVQSTYPGSTYASLNGTSMATPHVAGAAALVKQKNPSWSNVQIRNHLKNTATSLGSTNLYGSGLVNAEAATR

SEQ ID NO: 43 - protein, 275 aa, Bacillus amyloliquefaciens [sequence omitted]

SEQ ID NO: 44 - protein, 269 aa, Bacillus lentus
AQSVPWGISRVQAPAAHNRGLTGSGVKVAVLDTGISTHPDLNIRGGASFVPGEPSTQDGNGHGTHVAGTIAALNNSIGVLGVAPSAELYAVKVLGADGRGAISSIAQGLEWAGNNGMHVANLSLGSPSPSATLEQAVNSATSRGVLVVAASGNSGASSISYPARYANAMAVGATDQNNNRASFSQYGAGLDIVAPGVNVQSTYPGSTYASLNGTSMATPHVAGAAALVKQKNPSWSNVQIRNHLKNTATSLGSTNLYGSGLVNAEAATR

SEQ ID NO: 45 - protein, 434 aa, Bacillus sp.
NDVARGIVKADVAQSSYGLYGQGQIVAVADTGLDTGRNDSSMHEAFRGKITALYALGRTNNANDTNGHGTHVAGSVLGNGSTNKGMAPQANLVFQSIMDSGGGLGGLPSNLQTLFSQAYSAGARIHTNSWGAAVNGAYTTDSRNVDDYVRKNDMTILFAAGNEGPNGGTISAPGTAKNAITVGATENLRPSFGSYADNINHVAQFSSRGPTKDGRIKPDVMAPGTFILSARSSLAPDSSFWANHDSKYAYMGGTSMATPIVAGNVAQLREHFVKNRGITPKPSLLKAALIAGAADIGLGYPNGNQGWGRVTLDKSLNVAYVNESSSLSTSQKATYSFTATAGKPLKISLVWSDAPASTTASVTLVNDLDLVITAPNGTQYVGNDFTSPYNDNWDGRNNVENVFINAPQSGTYTIEVQAYNVPVGPQTFSLAIVN

SEQ ID NO: 46 - protein, 311 aa, Bacillus sp [sequence omitted]

SEQ ID NO: 47 - protein, 300 aa, Bacillus amyloliquefacience
AATTGTGTTLKGKTVSLNISSESGKYVLRDLSKPTGTQIITYDLQNREYNLPGTLVSSTTNQFTTSSQRAAVDAHYNLGKVYDYFYQKFNRNSYDNKGGKIVSSVHYGSRYNNAAWIGDQMIYGDGDGSFFSPLSGSMDVTAHEMTHGVTQETANLNYENQPGALNESFSDVFGYFNDTEDWDIGEDITVSQPALRSLSNPTKYGQPDNFKNYKNLPNTDAGDYGGVHTNSGIPNKAAYNTITKIGVNKAEQIYYRALTVYLTPSSTFKDAKAALIQSARDLYGSQDAASVEAAWNAVGL

SEQ ID NO: 48 - protein, 300 aa, Bacillus subtilis
AAATGSGTTLKGATVPLNISYEGGKYVLRDLSKPTGTQIITYDLQNRQSRLPGTLVSSTTKTFTSSSQRAAVDAHYNLGKVYDYFYSNFKRNSYDNKGSKIVSSVHYGTQYNNAAWTGDQMIYGDGDGSFFSPLSGSLDVTAHEMTHGVTQETANLIYENQPGALNESFSDVFGYFNDTEDWDIGEDITVSQPALRSLSNPTKYNQPDNYANYRNLPNTDEGDYGGVHTNSGIPNKAAYNTITKLGVSKSQQIYYRALTTYLTPSSTFKDAKAALIQSARDLYGSTDAAKVEAAWNAVGL